European Patent Application EP 4 640 836 A1, published October 29, 2025. Title: RECOMBINANT MICROORGANISM WITH REGULATED EXPRESSION OF ALKYL HYDROPEROXIDE REDUCTASE AND METHOD FOR PRODUCING O-PHOSPHOSERINE, CYSTEINE OR CYSTEINE DERIVATIVES USING THE SAME. Applicant: CJ CHEILJEDANG CORPORATION. Application KR. The sequence listing filed with the application follows.

SEQUENCE LISTING (37 sequences)

SEQ ID NO: 1 - protein, 187 aa, Escherichia sp.
MSLINTKIKPFKNQAFKNGEFIEITEKDTEGRWSVFFFYPADFTFVCPTELGDVADHYEELQKLGVDVYAVSTDTHFTHKAWHSSSETIAKIKYAMIGDPTGALTRNFDNMREDEGLADRATFVVDPQGIIQAIEVTAEGIGRDASDLLRKIKAAQYVASHPGEVCPAKWKEGEATLAPSLDLVGKI

SEQ ID NO: 2 - DNA, 564 bp, Escherichia coli
  source 1..564: mol_type = genomic DNA
atgtccttgattaacaccaaaattaaaccttttaaaaaccaggcattcaaaaacggcgaattcatcgaaatcaccgaaaaagataccgaaggccgctggagcgtcttcttcttctacccggctgactttactttcgtatgcccgaccgaactgggtgacgttgctgaccactacgaagaactgcagaaactgggcgtagacgtatacgcagtatctaccgatactcacttcacccacaaagcatggcacagcagctctgaaaccatcgctaaaatcaaatatgcgatgatcggcgacccgactggcgccctgacccgtaacttcgacaacatgcgtgaagatgaaggtctggctgaccgtgcgaccttcgttgttgacccgcagggtatcatccaggcaatcgaagttaccgctgaaggcattggccgtgacgcgtctgacctgctgcgtaaaatcaaagcagcacagtacgtagcttctcacccaggtgaagtttgcccggctaaatggaaagaaggtgaagcaactctggctccgtctctggacctggttggtaaaatctaa

SEQ ID NO: 3 - protein, 521 aa, Escherichia sp.
MLDTNMKTQLKAYLEKLTKPVELIATLDDSAKSAEIKELLAEIAELSDKVTFKEDNSLPVRKPSFLITNPGSNQGPRFAGSPLGHEFTSLVLALLWTGGHPSKEAQSLLEQIRHIDGDFEFETYYSLSCHNCPDVVQALNLMSVLNPRIKHTAIDGGTFQNEITDRNVMGVPAVFVNGKEFGQGRMTLTEIVAKIDTGAEKRAAEELNKRDAYDVLIVGSGPAGAAAAIYSARKGIRTGLMGERFGGQILDTVDIENYISVPKTEGQKLAGALKVHVDEYDVDVIDSQSASKLIPAAVEGGLHQIETASGAVLKARSIIVATGAKWRNMNVPGEDQYRTKGVTYCPHCDGPLFKGKRVAVIGGGNSGVEAAIDLAGIVEHVTLLEFAPEMKADQVLQDKLRSLKNVDIILNAQTTEVKGDGSKVVGLEYRDRVSGDIHNIELAGIFVQIGLLPNTNWLEGAVERNRMGEIIIDAKCETNVKGVFAAGDCTTVPYKQIIIATGEGAKASLSAFDYLIRTKTA

SEQ ID NO: 4 - DNA, 1566 bp, Escherichia coli
  source 1..1566: mol_type = genomic DNA
atgctcgacacaaatatgaaaactcaactcaaggcttaccttgagaaattgaccaagcctgttgagttaattgccacgctggatgacagcgctaaatcggcagaaatcaaggaactgttggctgaaatcgcagaactgtcagacaaagtcacctttaaagaagataacagcttgccggtgcgtaagccgtctttcctgatcaccaacccaggttccaaccaggggccacgttttgcaggctccccgctgggccacgagttcacctcgctggtactggcgttgctgtggaccggtggtcatccgtcgaaagaagcgcagtctctgctggagcagattcgccatattgacggtgattttgaattcgaaacctattactcgctctcttgccacaactgcccggacgtggtgcaggcgctgaacctgatgagcgtactgaacccgcgcatcaagcacactgcaattgacggcggcaccttccagaacgaaatcaccgatcgcaacgtgatgggcgttccggcagtgttcgtaaacgggaaagagtttggtcagggccgcatgacgttgactgaaatcgttgccaaaattgatactggcgcggaaaaacgtgcggcagaagagctgaacaagcgtgatgcttatgacgtattaatcgtcggttccggcccggcgggtgcagcggcagcaatttactccgcacgtaaaggcatccgtaccggtctgatgggcgaacgttttggtggtcagatcctcgataccgttgatatcgaaaactacatttctgtaccgaagactgaagggcagaagctggcaggcgcactgaaagttcacgttgatgaatacgacgttgatgtgatcgacagccagagcgccagcaaactgatcccagcagcagttgaaggtggtctgcatcagattgaaacagcttctggcgcggtactgaaagcacgcagcattatcgtggcgaccggtgcaaaatggcgcaacatgaacgttccgggcgaagatcagtatcgcaccaaaggcgtgacctactgcccgcactgcgacggcccgctgtttaaaggtaaacgcgtagcggttatcggcggcggtaactccggcgtggaagcggcaattgacctggcgggtatcgttgagcacgtaacgctgctggaatttgcgccagaaatgaaagccgaccaggttctgcaggacaaactgcgcagcctgaaaaacgtcgacattattctgaatgcgcaaaccacggaagtgaaaggcgacggcagcaaagtcgttggtctggaatatcgagatcgtgtcagcggcgatattcacaacatcgaactggccggtattttcgtccagattggtctgctgccgaacaccaactggctcgaaggcgcagtcgaacgtaaccgcatgggcgagattatcattgatgcgaaatgcgaaaccaacgtgaaaggcgtgttcgcagcgggtgactgtacgacggttccgtacaagcagatcatcatcgccactggcgaaggtgccaaagcctctctgagtgcttttgactacctgattcgcaccaaaactgcataa

SEQ ID NO: 5 - protein, 322 aa, unidentified [sequence omitted]

SEQ ID NO: 6 - DNA, 969 bp, unidentified
  source 1..969: mol_type = genomic DNA
atgcctaacattacctggtgcgacctgcctgaagatgtctctttatggccgggtctgcctctttcattaagtggtgatgaagtgatgccactggattaccacgcaggtcgtagcggctggctgctgtatggtcgtgggctggataaacaacgtctgacccaataccagagcaaactgggtgcggcgatggtgattgttgccgcctggtgcgtggaagattatcaggtgattcgtctggcaggttcactcaccgcacgggctacacgcctggcccacgaagcgcagctggatgtcgccccgctggggaaaatcccgcacctgcgcacgccgggtttgctggtgatggatatggactccaccgccatccagattgaatgtattgatgaaattgccaaactggccggaacgggcgagatggtggcggaagtaaccgaacgggcgatgcgcggcgaactcgattttaccgccagcctgcgcagccgtgtggcgacgctgaaaggcgctgacgccaatattctgcaacaggtgcgtgaaaatctgccgctgatgccaggcttaacgcaactggtgctcaagctggaaacgctgggctggaaagtggcgattgcctccggcggctttactttctttgctgaatacctgcgcgacaagctgcgcctgaccgccgtggtagccaatgaactggagatcatggacggtaaatttaccggcaatgtgatcggcgacatcgtagacgcgcagtacaaagcgaaaactctgactcgcctcgcgcaggagtatgaaatcccgctggcgcagaccgtggcgattggcgatggagccaatgacctgccgatgatcaaagcggcagggctggggattgcctaccatgccaagccaaaagtgaatgaaaaggcggaagtcaccatccgtcacgctgacctgatgggggtattctgcatcctctcaggcagcctgaatcagaagtaa

SEQ ID NO: 7 - protein, 405 aa, unidentified
MPEPVAEPALNGLRLNLRIVSIVMFNFASYLTIGLPLAVLPGYVHDVMGFSAFWAGLVISLQYFATLLSRPHAGRYADSLGPKKIVVFGLCGCFLSGLGYLTAGLTASLPVISLLLLCLGRVILGIGQSFAGTGSTLWGVGVVGSLHIGRVISWNGIVTYGAMAMGAPLGVVFYHWGGLQALALIIMGVALVAILLAIPRPTVKASKGKPLPFRAVLGRVWLYGMALALASAGFGVIATFITLFYDAKGWDGAAFALTLFSCAFVGTRLLFPNGINRIGGLNVAMICFSVEIIGLLLVGVATMPWMAKIGVLLAGAGFSLVFPALGVVAVKAVPQQNQGAALATYTVFMDLSLGVTGPLAGLVMSWAGVPVIYLAAAGLVAIALLLTWRLKKRPPEHVPEAASSS

SEQ ID NO: 8 - DNA, 1218 bp, unidentified
  source 1..1218: mol_type = genomic DNA
atgcccgaacccgtagccgaacccgcgctaaacggattgcgcctgaatttgcgcattgtctctatagtcatgtttaacttcgccagctacctcaccatcgggttgccgctcgctgtattaccgggctatgtccatgatgtgatgggctttagcgccttctgggcaggattggttatcagcctgcaatatttcgccaccttgctgagccgccctcatgccggacgttacgccgattcgctgggacccaaaaagattgtcgtcttcggtttatgcggctgctttttgagcggtctggggtatctgacggcaggattaaccgccagtctgcctgtcatcagcctgttattactttgcctggggcgcgtcatccttgggattgggcaaagttttgccggaacgggatcgaccctatggggcgttggcgtggttggctcgctgcatatcgggcgggtgatttcgtggaacggcattgtcacttacggggcgatggcgatgggtgcgccgttaggcgtcgtgttttatcactggggcggcttgcaggcgttagcgttaatcattatgggcgtggcgctggtggccattttgttggcgatcccgcgtccgacggtaaaagccagtaaaggcaaaccgctgccgtttcgcgcggtgcttgggcgcgtctggctgtacggtatggcgctggcactggcttccgccggatttggcgtcatcgccacctttatcacgctgttttatgacgctaaaggttgggacggtgcggctttcgcgctgacgctgtttagctgtgcgtttgtcggtacgcgtttgttattccctaacggcattaaccgtatcggtggcttaaacgtagcgatgatttgctttagcgttgagataatcggcctgctactggttggcgtggcgactatgccgtggatggcgaaaatcggcgtcttactggcgggggccgggttttcgctggtgttcccggcattgggtgtagtggcggtaaaagcggttccgcagcaaaatcagggggcggcgctggcaacttacaccgtatttatggatttatcgcttggcgtgactggaccactggctgggctggtgatgagctgggcgggcgtaccggtgatttatctggcggcggcgggactggtcgcaatcgcgttattactgacgtggcgattaaaaaaacggcctccggaacacgtccctgaggccgcctcatcatcttaa

SEQ ID NO: 9 - DNA, 300 bp, synthetic construct
  source 1..300: mol_type = other DNA
caggaagccgcttctattgcacaagagataaagcgtctaccttaattataaagatttgtaaatataaccgtctccggtatgttgcctgaggcggtttttttgtctctaacgtgcggaaaaatttgttcctcttcacattttttgtacaaccgacatgcccgtgtagctcacaaatatgacagtggcgtgaattttgcgcattgacggcagttatgattcgcggtattgcttaactgtgattgcacatttagtaatcactgttttcttttccaccagaaaccagtatgagggaaacgaggc

SEQ ID NO: 10 - DNA, 312 bp, synthetic construct
  source 1..312: mol_type = other DNA
gcctgtattcgttgtagtgaaatcattcatatgaaagcgggggaaaaacaattatgtccgcgctgtgcaaatccagaatggacgaaggcaagtcgggcaaaacgggtgacctgacagtaaaaacatcggctttttgctaataatccgagagattcttttgtgtgatgcaagccacatttttgccctcaacggttttactcattgcgatgtgtgtcactgaatgataaaaccgatagccacaggaataatgtattacctgtggtcgcaatcgattgaccgcgggttaatagcaacgcaacgtggtgaggggaa

SEQ ID NO: 11 - DNA, 35 bp, synthetic construct
  source 1..35: mol_type = other DNA
ctgcaggaattcgatgaaggtaaccactttttccg

SEQ ID NO: 12 - DNA, 35 bp, synthetic construct
  source 1..35: mol_type = other DNA
gagttgcagcaagcggaggatcaccacatttttac

SEQ ID NO: 13 - DNA, 35 bp, synthetic construct
  source 1..35: mol_type = other DNA
aatgtggtgatcctccgcttgctgcaactctctca

SEQ ID NO: 14 - DNA, 35 bp, synthetic construct
  source 1..35: mol_type = other DNA
tacgggttcgggcatgatagctctcctgtgtgaaa

SEQ ID NO: 15 - DNA, 35 bp, synthetic construct
  source 1..35: mol_type = other DNA
cacaggagagctatcatgcccgaacccgtagccga

SEQ ID NO: 16 - DNA, 35 bp, synthetic construct
  source 1..35: mol_type = other DNA
gtcgactagcgtgatagcggtttgcctttactggc

SEQ ID NO: 17 - DNA, 20 bp, synthetic construct
  source 1..20: mol_type = other DNA
agttgagcaaaaacgccagt

SEQ ID NO: 18 - DNA, 20 bp, synthetic construct
  source 1..20: mol_type = other DNA
gccataccgtacagccagac

SEQ ID NO: 19 - DNA, 36 bp, synthetic construct
  source 1..36: mol_type = other DNA
gctgcaggaattcgattccatcagtttctcattgtc

SEQ ID NO: 20 - DNA, 35 bp, synthetic construct
  source 1..35: mol_type = other DNA
gaagcggcttcctgctatacttcctccgtgttttc

SEQ ID NO: 21 - DNA, 35 bp, synthetic construct
  source 1..35: mol_type = other DNA
tgagggaaacgaggcatgtccttgattaacaccaa

SEQ ID NO: 22 - DNA, 35 bp, synthetic construct
  source 1..35: mol_type = other DNA
gtcgactagcgtgatcaaggcggctagcctgtgaa

SEQ ID NO: 23 - DNA, 35 bp, synthetic construct
  source 1..35: mol_type = other DNA
acggaggaagtatagcaggaagccgcttctattgc

SEQ ID NO: 24 - DNA, 36 bp, synthetic construct
  source 1..36: mol_type = other DNA
tgttaatcaaggacatgcctcgtttccctcatactg

SEQ ID NO: 25 - DNA, 35 bp, synthetic construct
  source 1..35: mol_type = other DNA
caacgaatacaggcctatacttcctccgtgttttc

SEQ ID NO: 26 - DNA, 35 bp, synthetic construct
  source 1..35: mol_type = other DNA
acgtggtgaggggaaatgtccttgattaacaccaa

SEQ ID NO: 27 - DNA, 35 bp, synthetic construct
  source 1..35: mol_type = other DNA
acggaggaagtataggcctgtattcgttgtagtga

SEQ ID NO: 28 - DNA, 35 bp, synthetic construct
  source 1..35: mol_type = other DNA
taatcaaggacatttcccctcaccacgttgcgttg

SEQ ID NO: 29 - DNA, 35 bp, synthetic construct
  source 1..35: mol_type = other DNA
atcatcgaccatcgctatacttcctccgtgttttc

SEQ ID NO: 30 - DNA, 44 bp, synthetic construct
  source 1..44: mol_type = other DNA
caccgggagttcatcatgtccttgattaacaccaaaattaaacc

SEQ ID NO: 31 - DNA, 42 bp, synthetic construct
  source 1..42: mol_type = other DNA
acggaggaagtatagcgatggtcgatgattaagacatcaaac

SEQ ID NO: 32 - DNA, 34 bp, synthetic construct
  source 1..34: mol_type = other DNA
gttaatcaaggacatgatgaactcccggtgtgtc

SEQ ID NO: 33 - DNA, 20 bp, synthetic construct
  source 1..20: mol_type = other DNA
atattaagcgttttctgatc

SEQ ID NO: 34 - DNA, 20 bp, synthetic construct
  source 1..20: mol_type = other DNA
ttctttcgacggatgaccac

SEQ ID NO: 35 - DNA, 379 bp, synthetic construct
  source 1..379: mol_type = other DNA
cgatggtcgatgattaagacatcaaaccccaaatggaacaggtcataggccagttccgcatattttacgtagctctcaatacgccccgggcagatgactaccacccggtcatggtgctgtgcgcgaaaacggacaaagcgcaccggaatgtcatccacaccagtaaactctgcttcatcacgctgacgccagaaatcagtcagcggtcccatggtaaaagcagcaaacgcgttttctcttgtttcccagtctttttgctgctgaaacatcgggtaatctgcctcttaaaccacgtaaaatcgttttttttagcgtgcctgacacaacgctgcgacagtagcgtattgtggcacaaaaatagacacaccgggagttcatc

SEQ ID NO: 36 - DNA, 4695 bp, synthetic construct
  source 1..4695: mol_type = other DNA
tcgaggccgcgattaaattccaacatggatgctgatttatatgggtataaatgggctcgcgataatgtcgggcaatcaggtgcgacaatctatcgattgtatgggaagcccgatgcgccagagttgtttctgaaacatggcaaaggtagcgttgccaatgatgttacagatgagatggtcagactaaactggctgacggaatttatgcctcttccgaccatcaagcattttatccgtactcctgatgatgcatggttactcaccactgcgatccccgggaaaacagcattccaggtattagaagaatatcctgattcaggtgaaaatattgttgatgcgctggcagtgttcctgcgccggttgcattcgattcctgtttgtaattgtccttttaacagcgatcgcgtatttcgtctcgctcaggcgcaatcacgaatgaataacggtttggttgatgcgagtgattttgatgacgagcgtaatggctggcctgttgaacaagtctggaaagaaatgcataagcttttgccattctcaccggattcagtcgtcactcatggtgatttctcacttgataaccttatttttgacgaggggaaattaataggttgtattgatgttggacgagtcggaatcgcagaccgataccaggatcttgccatcctatggaactgcctcggtgagttttctccttcattacagaaacggctttttcaaaaatatggtattgataatcctgatatgaataaattgcagtttcatttgatgctcgatgagtttttctaatcagaattggttaattggttgtaacactggcagagcattacgctgacttgacgggacggcggctttgttgaataaatcgaacttttgctgagttgaaggatcagatcacgcatcttcccgacaacgcagaccgttccgtggcaaagcaaaagttcaaaatcaccaactggtccacctacaacaaagctctcatcaaccgtggctccctcactttctggctggatgatggggcgattcaggcctggtatgagtcagcaacaccttcttcacgaggcagacctcagcgctcaaagatgcaggggtaaaagctaaccgcatctttaccgacaaggcatccggcagttcaacagatcgggaagggctggatttgctgaggatgaaggtggaggaaggtgatgtcattctggtgaagaagctcgaccgtcttggccgcgacaccgccgacatgatccaactgataaaagagtttgatgctcagggtgtagcggttcggtttattgacgacgggatcagtaccgacggtgatatggggcaaatggtggtcaccgcgcgtaatacgactcactatagggcgaattggagctccaccgcggtggcggccgctctagactttacggtatcgccgctcccgattcgcagcgcatcgccttctatcgccttcttgacgagttcttctgagcgggactctggggttcgctagaggatcgatcctttttaacccatcacatatacctgccgttcactattatttagtgaaatgagatattatgatattttctgaattgtgattaaaaaggcaactttatgcccatgcaacagaaactataaaaaatacagagaatgaaaagaaacagatagattttttagttctttaggcccgtagtctgcaaatccttttatgattttctatcaaacaaaagaggaaaatagaccagttgcaatccaaacgagagtctaatagaatgaggtcgaaaagtaaatcgcgcgggtttgttactgataaagcaggcaagacctaaaatgtgtaaagggcaaagtgtatactttggcgtcaccccttacatattttaggtctttttttattgtgcgtaactaacttgccatcttcaaacaggagggctggaagaagcagaccgctaacacagtacataaaaaaggagacatgaacgatgaacatcaaaaagtttgcaaaacaagcaacagtattaacctttactaccgcactgctggcaggaggcgcaactcaagcgtttgcgaaagaaacgaaccaaaagccatataaggaaacatacggcatttcccatattacacgccatgatatgctgcaaatccctgaacagcaaaaaaatgaaaaatatcaagttcctgaattcgattcgtccacaattaaaaatatctcttctgcaaaaggcctggacgtttgggacagctggccattacaaaacgctgacggcactgtcgcaaactatcacggctaccacatcgtctttgcattagccggagatcctaaaaatgcggatgacacatcgatttacatgttctatcaaaaagtcggcgaaacttctattgacagctggaaaaacgctggccgcgtctttaaagacagcgacaaattcgatgcaaatgattctatcctaaaagaccaaacacaagaatggtcaggttcagccacatttacatctgacggaaaaatccgtttattctacactgatttctccggtaaacattacggcaaacaaacactgacaactgcacaagttaacgtatcagcatcagacagctctttgaacatcaacggtgtagaggattataaatcaatctttgacggtgacggaaaaacgtatcaaaatgtacagcagttcatcgatgaaggcaactacagctcaggcgacaaccatacgctgagagatcctcactacgtagaagataaaggccacaaatacttagtatttgaagcaaacactggaactgaagatggctaccaaggcgaagaatctttatttaacaaagcatactatggcaaaagcacatcattcttccgtcaagaaagtcaaaaacttctgcaaagcgataaaaaacgcacggctgagttagcaaacggcgctctcggtatgattgagctaaacgatgattacacactgaaaaaagtgatgaaaccgctgattgcatctaacacagtaacagatgaaattgaacgcgcgaacgtctttaaaatgaacggcaaatggtacctgttcactgactcccgcggatcaaaaatgacgattgacggcattacgtctaacgatatttacatgcttggttatgtttctaattctttaactggcccatacaagccgctgaacaaaactggccttgtgttaaaaatggatcttgatcctaacgatgtaacctttacttactcacacttcgctgtacctcaagcgaaaggaaacaatgtcgtgattacaagctatatgacaaacagaggattctacgcagacaaacaatcaacgtttgcgccaagcttcctgctgaacatcaaaggcaagaaaacatctgttgtcaaagacagcatccttgaacaaggacaattaacagttaacaaataaaaacgcaaaagaaaatgccgatgggtaccgagcgaaatgaccgaccaagcgacgcccaacctgccatcggatcccccgggctgcaggaattcgatatcacgctagtcgacctagctagcatatggggagatctactagtaaagcatgccaattggtattctatagtgtcacctaaatcgtatgtgtatgatacataaggttatgtattaattgtagccgcgttctaacgacaatatgtacaagcctaattgtgtagcatctggcttactgaagcagaccctatcatctctctcgtaaactgccgtcagagtcggtttggttggacgaaccttctgagtttctggtaacgccgtcccgcacccggaaatggtcagcgaaccaatcagcagggtcatcgctagcccatggctaattcccatgtcagccgttaagtgttcctgtgtcactcaaaattgctttgagaggctctaagggcttctcagtgcgttacatccctggcttgttgtccacaaccgttaaaccttaaaagctttaaaagccttatatattcttttttttcttataaaacttaaaaccttagaggctatttaagttgctgatttatattaattttattgttcaaacatgagagcttagtacgtgaaacatgagagcttagtacgttagccatgagagcttagtacgttagccatgagggtttagttcgttaaacatgagagcttagtacgttaaacatgagagcttagtacgtgaaacatgagagcttagtacgtactatcaacaggttgaactgctgatcttcagatcctctacgccggacgcatcgtggccggatcttgcggccgcaaaaattaaaaatgaagttttaaatcaatctaaagtatatatgagtaaacttggtctgacagttaccaatgcttaatcagtgaggcaccaataactgccttaaaaaaactagcgctgaggtctgcctcgtgaagaaggtgttgctgactcataccaggcctgaatcgccccatcatccagccagaaagtgagggagccacggttgatgagagctttgttgtaggtggaccagttggtgattttgaacttttgctttgccacggaacggtctgcgttgtcgggaagatgcgtgatctgatccttcaactcagcaaaagttcgatttattcaacaaagccacgttgtgtctcaaaatctctgatgttacattgcacaagataaaaatatatcatcatgaacaataaaactgtctgcttacataaacagtaatacaaggggtgttatgagccatattcaacgggaaacgtcttgc

SEQ ID NO: 37 - DNA, 476 bp, synthetic construct
  source 1..476: mol_type = other DNA
cgcttgctgcaactctctcagggccaggcggtgaagggcaatcagctgttgcccgtctcactggtgaaaagaaaaaccaccctggcgcccaatacgcaaaccgcctctccccgcgcgttggccgattcattaatgcagctggcacgacaggtttcccgactggaaagcgggcagtgagcgcaacgcaattaatgtaagttagcgcgaattgatctggtttgacagcttatcatcgactgcacggtgcaccaatgcttctggcgtcaggcagccatcggaagctgtggtatggctgtgcaggtcgtaaatcactgcataattcgtgtcgctcaaggcgcactcccgttctggataatgttttttgcgccgacatcataacggttctggcaaatattctgaaatgagctgttgacaattaatcatccggctcgtataatgtgtggaattgtgagcggataacaatttcacacaggaaa